European Patent Application EP 4 338 749 A1, published March 20, 2024. Title: Vaccine against Helicobacter pylori infection. Applicant: IGUANA BioTechnology GmbH. Application EP. The sequence listing filed with the application follows.

SEQUENCE LISTING (36 sequences)

SEQ ID NO: 1 - protein, 16 aa, synthetic construct
GGGKTLREGMSQSNNP

SEQ ID NO: 2 - protein, 41 aa, synthetic construct
IEAGAIGFKIHEDWGTTPSAINHALDVADKYDVQVAIHTDT

SEQ ID NO: 3 - protein, 36 aa, synthetic construct
TLHDMGIFSITSSDSQAMGRVGEVITRTWQTADKNK

SEQ ID NO: 4 - protein, 23 aa, synthetic construct
SAINHALDVADKYDVQVAIHTDT

SEQ ID NO: 5 - protein, 23 aa, synthetic construct
QGDINELGAKFSSRDDIFSQVDT

SEQ ID NO: 6 - protein, 26 aa, synthetic construct
PKATQDFFYGSDSKDMGGREIHQEGI

SEQ ID NO: 7 - protein, 20 aa, synthetic construct
TGGNDPYQLMVNTKNTGEDN

SEQ ID NO: 8 - protein, 31 aa, synthetic construct
TNGEVMGIVMKTGGNDPYQLMVNTKNTGEDN

SEQ ID NO: 9 - protein, 10 aa, synthetic construct
TLLSSLKGPV

SEQ ID NO: 10 - protein, 31 aa, synthetic construct
SALNSNPKATQDFFYGSDSKDMGGREIHQEG

SEQ ID NO: 11 - protein, 11 aa, synthetic construct
TLLSSLKGPVK

SEQ ID NO: 12 - protein, 28 aa, synthetic construct
RSSLNNVFSYSVHTDNGVESLMKYGLSL

SEQ ID NO: 13 - protein, 10 aa, synthetic construct
TLLSSLKGPV

SEQ ID NO: 14 - protein, 15 aa, synthetic construct
GEVMGIVMKTGGNDP

SEQ ID NO: 15 - protein, 9 aa, synthetic construct
DDIFSQVDT

SEQ ID NO: 16 - protein, 25 aa, synthetic construct
DPKRTIQKKSEPGLLFSTGLDKMEG

SEQ ID NO: 17 - protein, 49 aa, synthetic construct
EPMSGESLDSFTMDLSELDIQEKFLKTTHSSHSGGLVSTMVKGTDNSND

SEQ ID NO: 18 - protein, 16 aa, synthetic construct
KVTILEPMSGESLDSF

SEQ ID NO: 19 - protein, 12 aa, synthetic construct
VLIPAGFIKVTI

SEQ ID NO: 20 - protein, 22 aa, synthetic construct
GESLDSFTMDLSELDIQEKFLK

SEQ ID NO: 21 - protein, 20 aa, synthetic construct
LTQKNLESYQKDAKELQNKR

SEQ ID NO: 22 - protein, 20 aa, synthetic construct
ALKVEQILQNQGYKVISVDS

SEQ ID NO: 23 - protein, 34 aa, synthetic construct
SANDKRMQDNLVSVIEKQTNKKVRILEIKPLKSS

SEQ ID NO: 24 - protein, 24 aa, synthetic construct
SVIEKQTNKKVRILEIKPLKSSQD

SEQ ID NO: 25 - protein, 17 aa, synthetic construct
TNKKVRILEIKPLKSSQ

SEQ ID NO: 26 - protein, 17 aa, synthetic construct
VVVGWLGVNSAKKAALI

SEQ ID NO: 27 - protein, 38 aa, synthetic construct
EEMAKARARGASVEDKISILEKIYSTQYDINAQKEPED

SEQ ID NO: 28 - protein, 13 aa, synthetic construct
QLGHHPLVTLSEA

SEQ ID NO: 29 - protein, 11 aa, synthetic construct
TRVKEETKTSF

SEQ ID NO: 30 - protein, 26 aa, synthetic construct
SAINTNEQSTPIGESGKNFNPFKDAS

SEQ ID NO: 31 - protein, 142 aa, synthetic construct
MAQVINTNSLSLLTQNNLNKSQSSLSSAIERLSSGLRINSAKDDAAGQAIANRFTSNIKGLTQASRNANDGISIAQTTEGALNEINNNLQRVRELSVQATNGTNSDSDLKSIQDEIQQRLEEIDRVSNQTQFNGVKVLSQDN

SEQ ID NO: 32 - protein, 87 aa, synthetic construct
LASIDSALSKVDAVRSSLGAIQNRFDSAITNLGNTVTNLNSVRSRIEDADYATEVSNMSKAQILQQAGTSVLAQANQVPQNVLSLLR

SEQ ID NO: 33 - protein, 505 aa, synthetic construct
MAQVINTNSLSLLTQNNLNKSQSSLSSAIERLSSGLRINSAKDDAAGQAIANRFTSNIKGLTQASRNANDGISIAQTTEGALNEINNNLQRVRELSVQATNGTNSDSDLKSIQDEIQQRLEEIDRVSNQTQFNGVKVLSQDNQMKIQVGANDGETITIDLQKIDVKSLGLDGFNVNGPKEATVGDLKSSFKNVTGYDTYAAGADKYRVDINSGAVVTDAAAPDKVYVNAANGQLTTDDAENNTAVNLFKTTKSTAGTDEAKAIAGAIKGGKEGDTFDYKGVSFTIDTKAGNDGNGTVSTTINGEKVTLTVADITAGAANVNDATLQSSKNVYTSVVNGQFTFDDKTKNESAKLSDLEANNAVKGESKITVNGAEYTANAAGDKVTLAGKTMFIDKTASGVSTLINEDAAAAKKSTANPLASIDSALSKVDAVRSSLGAIQNRFDSAITNLGNTVTNLNSVRSRIEDADYATEVSNMSKAQILQQAGTSVLAQANQVPQNVLSLLR

SEQ ID NO: 34 - protein, 106 aa, synthetic construct
MTPQNITDLCAEYHNTQIYTLNDKIFSYTESLAGKREMAIITFKNGAIFQVEVPGSQHIDSQKKAIERMKDTLRIAYLTEAKVEKLCVWNNKTPHAIAAISMANGT

SEQ ID NO: 35 - protein, 256 aa, synthetic construct
SITCSFNNLGIGYFGVMSIENMKKLNEAYQILQAALKQGLPALKENNGTIKDVTYSYICYGEGNNNCEIKLADGQKLQQNGGSETTTQTIDGKTVSTTISSKVVDSTAADNTYKQSYTEITNALKDVPDNAQALLAQASTLINTINTACPYFSVTNSSSPNAPKMEPTKGKLCGFTDEISAIQKMITDAQELVNQTSAINTNEQSTPIGESGKNFNPFKDASFAQGMLANASAQAKMLSLADQVGQAINPDRLTGN

SEQ ID NO: 36 - protein, 1068 aa, synthetic construct
CATATGATGGGAGATCGCCTGTATCGTGCTGATAGCCGTCCACCGGACGAAATCAAACGCTCGGGTGGCTTAATGCCGCGTGGTCATAACGAGTACTTTGATCGTGGTACGCAGATGAACATCAATCTGTATGACCACGCACGTGGCACACAAACTGGCTTCGTTCGGTATGACGATGGCTATGTCAGCACTTCGCTCTCGTTACGTTCTGCCCACTTAGCCGGCCAAAGCATTCTGAGCGGGTATAGCACGTATTACATCTACGTGATCGCTACTGCACCGAATATGTTCAACGTGAATGACGTGTTGGGCGTTTACAGTCCACATCCGTACGAACAGGAAGTTAGTGCGCTGGGAGGCATTCCGTACTCCCAGATCTATGGGTGGTATCGCGTCAACTTTGGGGTGATCGATGAACGGCTTCATCGCAATCGCGAGTATCGTGATCGTTACTACCGCAACCTGAACATTGCCCCAGCGGAAGATGGTTACCGCCTTGCCGGCTTTCCGCCGGATCATCAGGCATGGCGCGAAGAACCGTGGATTCACCATGCTCCCCAAGGCTGTGGCAATAGCAGTGGTACCATTACCGGGGACACGTGCAACGAAGAAACGCAAAATCTGTCGACAATTTACGCCCGTGAGTATCAGTCAAAAGTCAAACGCCAAATTTTCTCCGATTATCAGTCTGAAGTAGACATCTACAATCGCATTCGCGATGAACTCGGCGGTTCAGGTGGATCAGGTGGGAGTGCGCCTCAGACCATTACCGAGCTGTGTTCCGAGTATCGCAATACGCAGATTTATACGATCAACGACAAAATTCTGTCGTATACTGAGAGCATGGCGGGTAAACGCGAAATGGTGATTATCACCTTTAAAAGCGGTGAAACCTTTCAGGTTGAGGTACCTGGCTCTCAACACATCGATTCACAGAAGAAAGCGATTGAACGTATGAAAGATACCCTGCGCATTACCTATCTGACCGAAACCAAGATCGATAAATTGTGCGTGTGGAACAACAAAACACCCAACTCTATTGCAGCGATTTCCATGAAGAATCTCGAG